European Patent Specification EP 4 003 290 B1, published September 18, 2024. Title: STABILIZING THERAPEUTIC PROTEINS WITH PIPERAZIN- OR MORPHOLINE-CONTAINING ZWITTERIONIC BUFFERING SUBSTANCES. Applicant: HYpharm GmbH. Application not yet assigned. The sequence listing filed with the application follows.

SEQUENCE LISTING (6 sequences)

SEQ ID NO: 1 - protein, 163 aa, Bacteriophage phi-K
  CHAP domain of lysK
MAKTQAEINKRLDAYAKGTVDSPYRVKKATSYDPSFGVMEAGAIDADGYYHAQCQDLITDYVLWLTDNKVRTWGNAKDQIKQSYGTGFKIHENKPSTVPKKGWIAVFTSGSYEQWGHIGIVYDGGNTSTFTILEQNWNGYANKKPTKRVDNYYGLTHFIEIPV

SEQ ID NO: 2 - protein, 123 aa, Staphylococcus simulans
SNSTAQDPMPFLKSAGYGKAGGTVTPTPNTGWKTNKYGTLYKSESASFTPNTDIITRTTGPFRSMPQSGVLKAGQTIHYDEVMKQDGHVWVGYTGNSGQRIYLPVRTWNKSTNTLGVLWGTIK

SEQ ID NO: 3 - DNA, 489 bp, Bacteriophage phi-K
  CHAP domain of lysK
atggcgaaaacccaggcggaaattaacaaacgtctggatgcgtatgcgaaaggcaccgtggatagcccgtatcgtgtgaaaaaagcgaccagctatgatccgagctttggcgtgatggaagcgggtgcgattgatgcggatggctattatcacgcgcagtgccaggatctgattaccgattatgtgctgtggctgaccgataacaaagtgcgtacctggggcaacgcgaaagatcagatcaaacagagctatggcaccggctttaaaatccatgaaaacaaaccgagcaccgtgccgaaaaaaggctggattgcggtgtttaccagcggcagctatgaacagtggggccatattggcattgtgtatgatggcggcaacaccagcacctttaccattctggaacagaactggaacggctatgcgaacaaaaaaccgaccaaacgcgtggataactattatggcctgacccattttattgaaattccggtg

SEQ ID NO: 4 - DNA, 369 bp, Staphylococcus simulans
tctaatagcaccgcgcaggacccgatgccgttcttgaagtcggcgggctatggcaaagcaggcggcaccgtgactccgaccccgaacacgggctggaaaaccaacaagtacggtactctttacaaaagcgagagcgcatcttttacgccaaacacggacatcatcacgcgcaccaccggcccatttcgcagcatgccacagagcggcgtcttgaaagcgggccagaccattcactacgatgaagttatgaaacaggacggccatgtgtgggtgggctataccggcaacagcggccagcgtatttatttaccggttcgcacctggaataaaagcaccaataccttaggcgtgttatggggtaccattaag

SEQ ID NO: 5 - protein, 281 aa, Artificial Sequence
  Clone HY-133
MAKTQAEINKRLDAYAKGTVDSPYRVKKATSYDPSFGVMEAGAIDADGYYHAQCQDLITDYVLWLTDNKVRTWGNAKDQIKQSYGTGFKIHENKPSTVPKKGWIAVFTSGSYEQWGHIGIVYDGGNTSTFTILEQNWNGYANKKPTKRVDNYYGLTHFIEIPVGGSKPGGTKPGGSKPGSTVTPTPNTGWKTNKYGTLYKSESASFTPNTDIITRTTGPFRSMPQSGVLKAGQTIHYDEVMKQDGHVWVGYTGNSGQRIYLPVRTWNKSTNTLGVLWGTIK

SEQ ID NO: 6 - DNA, 846 bp, Artificial Sequence
  Clone HY-133
atggcgaaaacccaggcggaaattaacaaacgtctggatgcgtatgcgaaaggcaccgtggatagcccgtatcgtgtgaaaaaagcgaccagctatgatccgagctttggcgtgatggaagcgggtgcgattgatgcggatggctattatcacgcgcagtgccaggatctgattaccgattatgtgctgtggctgaccgataacaaagtgcgtacctggggcaacgcgaaagatcagatcaaacagagctatggcaccggctttaaaatccatgaaaacaaaccgagcaccgtgccgaaaaaaggctggattgcggtgtttaccagcggcagctatgaacagtggggccatattggcattgtgtatgatggcggcaacaccagcacctttaccattctggaacagaactggaacggctatgcgaacaaaaaaccgaccaaacgcgtggataactattatggcctgacccattttattgaaattccggtgggcggtagcaaacctggaggcacgaagccgggtggaagcaaaccaggatcgaccgtgactccgaccccgaacacgggctggaaaaccaacaagtacggtactctttacaaaagcgagagcgcatcttttacgccaaacacggacatcatcacgcgcaccaccggcccatttcgcagcatgccacagagcggcgtcttgaaagcgggccagaccattcactacgatgaagttatgaaacaggacggccatgtgtgggtgggctataccggcaacagcggccagcgtatttatttaccggttcgcacctggaataaaagcaccaataccttaggcgtgttatggggtaccattaagtaa